European Patent Application EP 4 477 268 A2, published December 18, 2024. Title: IMPROVED WOUND CARE DEVICE. Applicant: Amferia AB. Application EP. The sequence listing filed with the application follows.

SEQUENCE LISTING (5 sequences)

SEQ ID NO: 1 - protein, 13 aa, synthetic construct
  REGION 1..13: note = RRP9W4N synthetic peptide
  MOD_RES 13: note = AMIDATION
RRPRPRPRPWWWW

SEQ ID NO: 2 - protein, 9 aa, synthetic construct
  REGION 1..9: note = RRP9N synthetic peptide
  MOD_RES 9: note = AMIDATION
RRPRPRPRP

SEQ ID NO: 3 - protein, 9 aa, synthetic construct
  REGION 1..9: note = RRPRPRPRP synthetic peptide
RRPRPRPRP

SEQ ID NO: 4 - protein, 13 aa, synthetic construct
  REGION 1..13: note = RRPRPRPWWWWRP synthetic peptide
  MOD_RES 13: note = AMIDATION
RRPRPRPWWWWRP

SEQ ID NO: 5 - protein, 13 aa, synthetic construct
  REGION 1..13: note = RRP5W2RPW2RPN syntehtic peptide
  MOD_RES 13: note = AMIDATION
RRPRPWWRPWWRP